European Patent Application EP 4 212 633 A1, published July 19, 2023. Title: Molecules targeting viral RNA and/or viral RNA-protein complexes for use in the treatment of viral infections, in particular COVID-19. Applicant: Johann Wolfgang Goethe-Universität Frankfurt am Main Technische Universität Darmstadt. The sequence listing filed with the application follows.

SEQUENCE LISTING (3 sequences)

SEQ ID NO: 1 - RNA, 77 nt, artificial
  pseudoknot
ggccaguaggcgguguaagugcagcccgucuuacaccgugcggcacaggcacuaguacugaugucguauacagggcu

SEQ ID NO: 2 - DNA, 87 bp, artificial
  in-line probe
  Cy5 (1)..(1)
ttttttttttggccaguaggcgguguaagugcagcccgucuuacaccgugcggcacaggcacuaguacugaugucguauacagggcu

SEQ ID NO: 3 - RNA, 29 nt, artificial
  5_SL1 blocking sequence
ggguuuauaccuucccagguaacaaaccc